European Patent Application EP 4 796 180 A1, published August 26, 2026. Title: A therapeutic VHH antibody that blocks infection by herpes simplex viruses 1 and 2. Applicant: Max-Planck-Gesellschaft zur Foerderung der Wissenschaften e.V. The sequence listing filed with the application follows.

SEQUENCE LISTING (20 sequences)

SEQ ID NO: 1 - protein, 904 aa, Herpes simplex virus 1
  source 1..904: note = gB_HSV1 with signal peptide
  SIGNAL 1..30
  REGION 106: note = part of Nb1 epitope
  REGION 108: note = part of Nb1 epitope
  REGION 121..122: note = part of Nb1 epitope
  REGION 285..286: note = part of Nb1 epitope
  REGION 292: note = part of Nb1 epitope
  REGION 294: note = part of Nb1 epitope
  REGION 296: note = part of Nb1 epitope
  REGION 311..315: note = part of Nb1 epitope
  REGION 317: note = part of Nb1 epitope
  REGION 348..349: note = part of Nb1 epitope
  REGION 585: note = part of Nb1 epitope
  REGION 640: note = part of Nb1 epitope
  REGION 651: note = part of Nb1 epitope
  REGION 654..659: note = part of Nb1 epitope
  REGION 663: note = part of Nb1 epitope
MHQGAPSWGRRWFVVWALLGLTLGVLVASAAPTSPGTPGVAAATQAANGGPATPAPPPLGAAPTGDPKPKKNKKPKNPTPPRPAGDNATVAAGHATLREHLRDIKAENTDANFYVCPPPTGATVVQFEQPRRCPTRPEGQNYTEGIAVVFKENIAPYKFKATMYYKDVTVSQVWFGHRYSQFMGIFEDRAPVPFEEVIDKINAKGVCRSTAKYVRNNLETTAFHRDDHETDMELKPANAATRTSRGWHTTDLKYNPSRVEAFHRYGTTVNCIVEEVDARSVYPYDEFVLATGDFVYMSPFYGYREGSHTEHTSYAADRFKQVDGFYARDLTTKARATAPTTRNLLTTPKFTVAWDWVPKRPSVCTMTKWQEVDEMLRSEYGGSFRFSSDAISTTFTTNLTEYPLSRVDLGDCIGKDARDAMDRIFARRYNATHIKVGQPQYYLANGGFLIAYQPLLSNTLAELYVREHLREQSRKPPNPTPPPPGASANASVERIKTTSSIEFARLQFTYNHIQRHVNDMLGRVAIAWCELQNHELTLWNEARKLNPNAIASVTVGRRVSARMLGDVMAVSTCVPVAADNVIVQNSMRISSRPGACYSRPLVSFRYEDQGPLVEGQLGENNELRLTRDAIEPCTVGHRRYFTFGGGYVYFEEYAYSHQLSRADITTVSTFIDLNITMLEDHEFVPLEVYTRHEIKDSGLLDYTEVQRRNQLHDLRFADIDTVIHADANAAMFAGLGAFFEGMGDLGRAVGKVVMGIVGGVVSAVSGVSSFMSNPFGALAVGLLVLAGLAAAFFAFRYVMRLQSNPMKALYPLTTKELKNPTNPDASGEGEEGGDFDEAKLAEAREMIRYMALVSAMERTEHKAKKKGTSALLSAKVTDMVMRKRRNTNYTQVPNKDGDADEDDL

SEQ ID NO: 2 - protein, 904 aa, Herpes simplex virus 2
  source 1..904: note = gB_HSV-2 with signal peptide
  SIGNAL 1..22
  REGION 101: note = part of Nb1 epitope
  REGION 116..117: note = part of Nb1 epitope
  REGION 280..281: note = part of Nb1 epitope
  REGION 287: note = part of Nb1 epitope
  REGION 289: note = part of Nb1 epitope
  REGION 291: note = part of Nb1 epitope
  REGION 306..310: note = part of Nb1 epitope
  REGION 313: note = part of Nb1 epitope
  REGION 343: note = part of Nb1 epitope
  REGION 582: note = part of Nb1 epitope
  REGION 637: note = part of Nb1 epitope
  REGION 648: note = part of Nb1 epitope
  REGION 651..655: note = part of Nb1 epitope
  REGION 660: note = part of Nb1 epitope
MRGGGLICALVVGALVAAVASAAPAAPAAPRASGGVAATVAANGGPASRPPPVPSPATTKARKRKTKKPPKRPEATPPPDANATVAAGHATLRAHLREIKVENADAQFYVCPPPTGATVVQFEQPRRCPTRPEGQNYTEGIAVVFKENIAPYKFKATMYYKDVTVSQVWFGHRYSQFMGIFEDRAPVPFEEVIDKINAKGVCRSTAKYVRNNMETTAFHRDDHETDMELKPAKVATRTSRGWHTTDLKYNPSRVEAFHRYGTTVNCIVEEVDARSVYPYDEFVLATGDFVYMSPFYGYREGSHTEHTSYAADRFKQVDGFYARDLTTKARATSPTTRNLLTTPKFTVAWDWVPKRPAVCTMTKWQEVDEMLRAEYGGSFRFSSDAISTTFTTNLTQYSLSRVDLGDCIGRDAREAIDRMFARKYNATHIKVGQPQYYLATGGFLIAYQPLLSNTLAELYVREYMREQDRKPRNATPAPLREAPSANASVERIKTTSSIEFARLQFTYNHIQRHVNDMLGRIAVAWCELQNHELTLWNEARKLNPNAIASATVGRRVSARMLGDVMAVSTCVPVAPDNVIVQNSMRVSSRPGTCYSRPLVSFRYEDQGPLIEGQLGENNELRLTRDALEPCTVGHRRYFIFGGGYVYFEEYAYSHQLSRADVTTVSTFIDLNITMLEDHEFVPLEVYTRHEIKDSGLLDYTEVQRRNQLHDLRFADIDTVIRADANAAMFAGLCAFFEGMGDLGRAVGKVVMGVVGGVVSAVSGVSSFMSNPFGALAVGLLVLAGLVAAFFAFRYVLQLQRNPMKALYPLTTKELKTSDPGGVGGEGEEGAEGGGFDEAKLAEAREMIRYMALVSAMERTEHKARKKGTSALLSSKVTNMVLRKRNKARYSPLHNEDEAGDEDEL

SEQ ID NO: 3 - protein, 892 aa, synthetic construct
  source 1..892: note = HSV-1 gB used for primary immunization; note = based on UniProt P06437 (31-904) with Y889A point mutation
  REGION 875..892: note = linker and His-Tag
APTSPGTPGVAAATQAANGGPATPAPPPLGAAPTGDPKPKKNKKPKNPTPPRPAGDNATVAAGHATLREHLRDIKAENTDANFYVCPPPTGATVVQFEQPRRCPTRPEGQNYTEGIAVVFKENIAPYKFKATMYYKDVTVSQVWFGHRYSQFMGIFEDRAPVPFEEVIDKINAKGVCRSTAKYVRNNLETTAFHRDDHETDMELKPANAATRTSRGWHTTDLKYNPSRVEAFHRYGTTVNCIVEEVDARSVYPYDEFVLATGDFVYMSPFYGYREGSHTEHTSYAADRFKQVDGFYARDLTTKARATAPTTRNLLTTPKFTVAWDWVPKRPSVCTMTKWQEVDEMLRSEYGGSFRFSSDAISTTFTTNLTEYPLSRVDLGDCIGKDARDAMDRIFARRYNATHIKVGQPQYYLANGGFLIAYQPLLSNTLAELYVREHLREQSRKPPNPTPPPPGASANASVERIKTTSSIEFARLQFTYNHIQRHVNDMLGRVAIAWCELQNHELTLWNEARKLNPNAIASVTVGRRVSARMLGDVMAVSTCVPVAADNVIVQNSMRISSRPGACYSRPLVSFRYEDQGPLVEGQLGENNELRLTRDAIEPCTVGHRRYFTFGGGYVYFEEYAYSHQLSRADITTVSTFIDLNITMLEDHEFVPLEVYTRHEIKDSGLLDYTEVQRRNQLHDLRFADIDTVIHADANAAMFAGLGAFFEGMGDLGRAVGKVVMGIVGGVVSAVSGVSSFMSNPFGALAVGLLVLAGLAAAFFAFRYVMRLQSNPMKALYPLTTKELKNPTNPDASGEGEEGGDFDEAKLAEAREMIRYMALVSAMERTEHKAKKKGTSALLSAKVTDMVMRKRRNTNATQVPNKDGDADEDDLQLGSGSGSGSGSHHHHHH

SEQ ID NO: 4 - protein, 892 aa, synthetic construct
  source 1..892: note = HSV-1 gB used for immunogen production - additional boost; note = based on UniProt P06437 (31-904) with H516P and Y889A point mutations
  REGION 875..892: note = linker and His-Tag
APTSPGTPGVAAATQAANGGPATPAPPPLGAAPTGDPKPKKNKKPKNPTPPRPAGDNATVAAGHATLREHLRDIKAENTDANFYVCPPPTGATVVQFEQPRRCPTRPEGQNYTEGIAVVFKENIAPYKFKATMYYKDVTVSQVWFGHRYSQFMGIFEDRAPVPFEEVIDKINAKGVCRSTAKYVRNNLETTAFHRDDHETDMELKPANAATRTSRGWHTTDLKYNPSRVEAFHRYGTTVNCIVEEVDARSVYPYDEFVLATGDFVYMSPFYGYREGSHTEHTSYAADRFKQVDGFYARDLTTKARATAPTTRNLLTTPKFTVAWDWVPKRPSVCTMTKWQEVDEMLRSEYGGSFRFSSDAISTTFTTNLTEYPLSRVDLGDCIGKDARDAMDRIFARRYNATHIKVGQPQYYLANGGFLIAYQPLLSNTLAELYVREHLREQSRKPPNPTPPPPGASANASVERIKTTSSIEFARLQFTYNHIQRPVNDMLGRVAIAWCELQNHELTLWNEARKLNPNAIASVTVGRRVSARMLGDVMAVSTCVPVAADNVIVQNSMRISSRPGACYSRPLVSFRYEDQGPLVEGQLGENNELRLTRDAIEPCTVGHRRYFTFGGGYVYFEEYAYSHQLSRADITTVSTFIDLNITMLEDHEFVPLEVYTRHEIKDSGLLDYTEVQRRNQLHDLRFADIDTVIHADANAAMFAGLGAFFEGMGDLGRAVGKVVMGIVGGVVSAVSGVSSFMSNPFGALAVGLLVLAGLAAAFFAFRYVMRLQSNPMKALYPLTTKELKNPTNPDASGEGEEGGDFDEAKLAEAREMIRYMALVSAMERTEHKAKKKGTSALLSAKVTDMVMRKRRNTNATQVPNKDGDADEDDLQLGSGSGSGSGSHHHHHH

SEQ ID NO: 5 - protein, 924 aa, synthetic construct
  source 1..924: note = HSV-1 gB stabilised (31-904) used for structure determination
  REGION 875..924: note = linker and HRV3C protease site and StrepII tag
APTSPGTPGVAAATQAANGGPATPAPPPLGAAPTGDPKPKKNKKPKNPTPPRPAGDNATVAAGHATLREHLRDIKAENTDANFYVCPPPTGATVVQFEQPRRCPTRPEGQNYTEGIAVVFKENIAPYKFKATMYYKDVTVSQVWFGHRYSQFMGIFEDRAPVPFEEVIDKINAKGVCRSTAKYVRNNLETTAFHRDDHETDMELKPANAATRTSRGWHTTDLKYNPSRVEAFHRYGTTVNCIVEEVDARSVYPYDEFVLATGDFVYMSPFYGYREGSHTEHTSYAADRFKQVDGFYARDLTTKARATAPTTRNLLTTPKFTVAWDWVPKRPSVCTMTKWQEVDEMLRSEYGGSFRFSSDAICTTFTTNLTEYPLSRVDLGDCIGKDARDAMDRIFARRYNATHIKVGQPQYYLANGGFLIAYQPLLSNTLAELYVREHLREQSRKPPNPTPPPPGASANASVERIKTTSSIEFARLQFTYNHIQRPVNDMLGRVAIAWCELCNHELTLWNEARKLNPNAIASVTVGRRVSARMLGDVMAVSTCVPVAADNVIVQNSMRISSRPGACYSRPLVSFRYEDQGPLVEGQLGENNELRLTRDAIEPCTVGHRRYFTFGGGYVYFEEYAYSHQLSRADITTVSTFIDLNITMLEDHEFVPLEVYTRHEIKDSGLLDYTEVQRRVQLHDLRFADIDTVIHADANAAMFAGLGAFFEGMGDLGRAVGKVVMGIVGGVVSAVSGVSSFMSNPFGALAVGLLVLAGLAAAFFAFRYVMRLQSNPMKALYPLTTKELKNPTNPDASGEGEEGGDFDEAKLAEAREMIRYMALVSAMERTEHKAKKKGTSALLSAKVTDMVMRKRRNTNYTQVPNKDGDADEDDLQLGSGSGTLEVLFQGPGGSGSAWSHPQFEKGGGSGGGSGGSAWSHPQFEK

SEQ ID NO: 6 - protein, 926 aa, synthetic construct
  source 1..926: note = HSV-2 gB used for structure determination; note = based on UniProt P06763 (23-904)
  REGION 883..926: note = linker and HRV3C protease site and StrepII tag
APAAPAAPRASGGVAATVAANGGPASRPPPVPSPATTKARKRKTKKPPKRPEATPPPDANATVAAGHATLRAHLREIKVENADAQFYVCPPPTGATVVQFEQPRRCPTRPEGQNYTEGIAVVFKENIAPYKFKATMYYKDVTVSQVWFGHRYSQFMGIFEDRAPVPFEEVIDKINAKGVCRSTAKYVRNNMETTAFHRDDHETDMELKPAKVATRTSRGWHTTDLKYNPSRVEAFHRYGTTVNCIVEEVDARSVYPYDEFVLATGDFVYMSPFYGYREGSHTEHTSYAADRFKQVDGFYARDLTTKARATSPTTRNLLTTPKFTVAWDWVPKRPAVCTMTKWQEVDEMLRAEYGGSFRFSSDAISTTFTTNLTQYSLSRVDLGDCIGRDAREAIDRMFARKYNATHIKVGQPQYYLATGGFLIAYQPLLSNTLAELYVREYMREQDRKPRNATPAPLREAPSANASVERIKTTSSIEFARLQFTYNHIQRHVNDMLGRIAVAWCELQNHELTLWNEARKLNPNAIASATVGRRVSARMLGDVMAVSTCVPVAPDNVIVQNSMRVSSRPGTCYSRPLVSFRYEDQGPLIEGQLGENNELRLTRDALEPCTVGHRRYFIFGGGYVYFEEYAYSHQLSRADVTTVSTFIDLNITMLEDHEFVPLEVYTRHEIKDSGLLDYTEVQRRNQLHDLRFADIDTVIRADANAAMFAGLCAFFEGMGDLGRAVGKVVMGVVGGVVSAVSGVSSFMSNPFGALAVGLLVLAGLVAAFFAFRYVLQLQRNPMKALYPLTTKELKTSDPGGVGGEGEEGAEGGGFDEAKLAEAREMIRYMALVSAMERTEHKARKKGTSALLSSKVTNMVLRKRNKARYSPLHNEDEAGDEDELGTLEVLFQGPGGSGSAWSHPQFEKGGGSGGGSGGSAWSHPQFEK

SEQ ID NO: 7 - protein, 1118 aa, synthetic construct
  source 1..1118: note = based on UniProt P06437 (31-904) and GenBank MH644049.1 2-238; note = HSV-1 gB-sfEGFP used as transfected GFP-fusion
  REGION 1..874: note = HSV-1 gB (31-904)
  REGION 882..1118: note = sfEGFP (2-238)
APTSPGTPGVAAATQAANGGPATPAPPALGAAPTGDPKPKKNKKPKNPTPPRPAGDNATVAAGHATLREHLRDIKAENTDANFYVCPPPTGATVVQFEQPRRCPTRPEGQNYTEGIAVVFKENIAPYKFKATMYYKDVTVSQVWFGHRYSQFMGIFEDRAPVPFEEVIDKINAKGVCRSTAKYVRNNLETTAFHRDDHETDMELKPANAATRTSRGWHTTDLKYNPSRVEAFHRYGTTVNCIVEEVDARSVYPYDEFVLATGDFVYMSPFYGYREGSHTEHTSYAADRFKQVDGFYARDLTTKARATAPTTRNLLTTPKFTVAWDWVPKRPSVCTMTKWQEVDEMLRSEYGGSFRFSSDAISTTFTTNLTEYPLSRVDLGDCIGKDARDAMDRIFARRYNATHIKVGQPQYYLANGGFLIAYQPLLSNTLAELYVREHLREQSRKPPNPTPPPPGASANASVERIKTTSSIEFARLQFTYNHIQRHVNDMLGRVAIAWCELQNHELTLWNEARKLNPNAIASVTVGRRVSARMLGDVMAVSTCVPVAADNVIVQNSMRISSRPGACYSRPLVSFRYEDQGPLVEGQLGENNELRLTRDAIEPCTVGHRRYFTFGGGYVYFEEYAYSHQLSRADITTVSTFIDLNITMLEDHEFVPLEVYTRHEIKDSGLLDYTEVQRRNQLHDLRFADIDTVIHADANAAMFAGLGAFFEGMGDLGRAVGKVVMGIVGGVVSAVSGVSSFMSNPFGALAVGLLVLAGLAAAFFAFRYVMRLQSNPMKALYPLTTKELKNPTNPDASGEGEEGGDFDEAKLAEAREMIRYMALVSAMERTEHKAKKKGTSALLSAKVTDMVMRKRRNTNYTQVPNKDGDADEDDLGTGSSGVSKGEELFTGVVPILVELDGDVNGHKFSVRGEGEGDATNGKLTLKFICTTGKLPVPWPTLVTTLTYGVQCFSRYPDHMKQHDFFKSAMPEGYVQERTISFKDDGTYKTRAEVKFEGDTLVNRIELKGIDFKEDGNILGHKLEYNFNSHNVYITADKQKNGIKANFKIRHNVEDGSVQLADHYQQNTPIGDGPVLLPDNHYLSTQSKLSKDPNEKRDHMVLLEFVTAAGITLGMDELYK

SEQ ID NO: 8 - protein, 1126 aa, synthetic construct
  source 1..1126: note = based on Uniprot P06763 (23-904) and GenBank MH644049.1 (2-238); note = HSV-2 gB-sfEGFP used as transfected GFP-fusion
  REGION 1..882: note = HSV-2 gB (23-904)
  REGION 890..1126: note = sfEGFP (2-238)
APAAPAAPRASGGVAATVAANGGPASRPPPVPSPATTKARKRKTKKPPKRPEATPPPDANATVAAGHATLRAHLREIKVENADAQFYVCPPPTGATVVQFEQPRRCPTRPEGQNYTEGIAVVFKENIAPYKFKATMYYKDVTVSQVWFGHRYSQFMGIFEDRAPVPFEEVIDKINAKGVCRSTAKYVRNNMETTAFHRDDHETDMELKPAKVATRTSRGWHTTDLKYNPSRVEAFHRYGTTVNCIVEEVDARSVYPYDEFVLATGDFVYMSPFYGYREGSHTEHTSYAADRFKQVDGFYARDLTTKARATSPTTRNLLTTPKFTVAWDWVPKRPAVCTMTKWQEVDEMLRAEYGGSFRFSSDAISTTFTTNLTQYSLSRVDLGDCIGRDAREAIDRMFARKYNATHIKVGQPQYYLATGGFLIAYQPLLSNTLAELYVREYMREQDRKPRNATPAPLREAPSANASVERIKTTSSIEFARLQFTYNHIQRHVNDMLGRIAVAWCELQNHELTLWNEARKLNPNAIASATVGRRVSARMLGDVMAVSTCVPVAPDNVIVQNSMRVSSRPGTCYSRPLVSFRYEDQGPLIEGQLGENNELRLTRDALEPCTVGHRRYFIFGGGYVYFEEYAYSHQLSRADVTTVSTFIDLNITMLEDHEFVPLEVYTRHEIKDSGLLDYTEVQRRNQLHDLRFADIDTVIRADANAAMFAGLCAFFEGMGDLGRAVGKVVMGVVGGVVSAVSGVSSFMSNPFGALAVGLLVLAGLVAAFFAFRYVLQLQRNPMKALYPLTTKELKTSDPGGVGGEGEEGAEGGGFDEAKLAEAREMIRYMALVSAMERTEHKARKKGTSALLSSKVTNMVLRKRNKARYSPLHNEDEAGDEDELGTGSSGVSKGEELFTGVVPILVELDGDVNGHKFSVRGEGEGDATNGKLTLKFICTTGKLPVPWPTLVTTLTYGVQCFSRYPDHMKQHDFFKSAMPEGYVQERTISFKDDGTYKTRAEVKFEGDTLVNRIELKGIDFKEDGNILGHKLEYNFNSHNVYITADKQKNGIKANFKIRHNVEDGSVQLADHYQQNTPIGDGPVLLPDNHYLSTQSKLSKDPNEKRDHMVLLEFVTAAGITLGMDELYK

SEQ ID NO: 9 - protein, 1105 aa, synthetic construct
  source 1..1105: note = based on (Uniprot Q4JR05 (72-931) and GenBank MH644049.1 (2-238); note = VZV gB-sfEGFP used as transfected GFP-fusion
  REGION 1..860: note = VZV gB (72-931)
  REGION 869..1105: note = sfEGFP (2-238)
VSPSSFYESLQVEPTQSEDITRSAHLGDGDEIREAIHKSQDAETKPTFYVCPPPTGSTIVRLEPPRTCPDYHLGKNFTEGIAVVYKENIAAYKFKATVYYKDVIVSTAWAGSSYTQITNRYADRVPIPVSEITDTIDKFGKCSSKATYVRNNHKVEAFNEDKNPQDMPLIASKYNSVGSKAWHTTNDTYMVAGTPGTYRTGTSVNCIIEEVEARSIFPYDSFGLSTGDIIYMSPFFGLRDGAYREHSNYAMDRFHQFEGYRQRDLDTRALLEPAARNFLVTPHLTVGWNWKPKRTEVCSLVKWREVEDVVRDEYAHNFRFTMKTLSTTFISETNEFNLNQIHLSQCVKEEARAIINRIYTTRYNSSHVRTGDIQTYLARGGFVVVFQPLLSNSLARLYLQELVRENTNHSPQKHPTRNTRSRRSVPVELRANRTITTTSSVEFAMLQFTYDHIQEHVNEMLARISSSWCQLQNRERALWSGLFPINPSALASTILDQRVKARILGDVISVSNCPELGSDTRIILQNSMRVSGSTTRCYSRPLISIVSLNGSGTVEGQLGTDNELIMSRDLLEPCVANHKRYFLFGHHYVYYEDYRYVREIAVHDVGMISTYVDLNLTLLKDREFMPLQVYTRDELRDTGLLDYSEIQRRNQMHSLRFYDIDKVVQYDSGTAIMQGMAQFFQGLGTAGQAVGHVVLGATGALLSTVHGFTTFLSNPFGALAVGLLVLAGLVAAFFAYRYVLKLKTSPMKALYPLTTKGLKQLPEGMDPFAEKPNATDTPIEEIGDSQNTEPSVNSGFDPDKFREAQEMIKYMTLVSAAERQESKARKKNKTSALLTSRLTGLALRNRRGYSRVRTENVTGVSGTGSSGVSKGEELFTGVVPILVELDGDVNGHKFSVRGEGEGDATNGKLTLKFICTTGKLPVPWPTLVTTLTYGVQCFSRYPDHMKQHDFFKSAMPEGYVQERTISFKDDGTYKTRAEVKFEGDTLVNRIELKGIDFKEDGNILGHKLEYNFNSHNVYITADKQKNGIKANFKIRHNVEDGSVQLADHYQQNTPIGDGPVLLPDNHYLSTQSKLSKDPNEKRDHMVLLEFVTAAGITLGMDELYK

SEQ ID NO: 10 - protein, 1127 aa, synthetic construct
  source 1..1127: note = HCMV gB-sfEGFP used as transfected GFP-fusion; note = based on Uniprot F5HB53 (25-907) and GenBank MH644049.1 (2-238)
  REGION 1..883: note = HCMB gB (25-907)
  REGION 891..1127: note = sfEGFP (2-238)
SSSTRGTSATHSHHSSHTTSAAHSRSGSVSQRVTSSQTVSHGVNETIYNTTLKYGDVVGVNTTKYPYRVCSMAQGTDLIRFERNIVCTSMKPINEDLDEGIMVVYKRNIVAHTFKVRVYQKVLTFRRSYAYIHTTYLLGSNTEYVAPPMWEIHHINSHSQCYSSYSRVIAGTVFVAYHRDSYENKTMQLMPDDYSNTHSTRYVTVKDQWHSRGSTWLYRETCNLNCMVTITTARSKYPYHFFATSTGDVVDISPFYNGTNRNASYFGENADKFFIFPNYTIVSDFGRPNSALETHRLVAFLERADSVISWDIQDEKNVTCQLTFWEASERTIRSEAEDSYHFSSAKMTATFLSKKQEVNMSDSALDCVRDEAINKLQQIFNTSYNQTYEKYGNVSVFETTGGLVVFWQGIKQKSLVELERLANRSSLNLTHNRTKRSTDGNNATHLSNMESVHNLVYAQLQFTYDTLRGYINRALAQIAEAWCVDQRRTLEVFKELSKINPSAILSAIYNKPIAARFMGDVLGLASCVTINQTSVKVLRDMNVKESPGRCYSRPVVIFNFANSSYVQYGQLGEDNEILLGNHRTEECQLPSLKIFIAGNSAYEYVDYLFKRMIDLSSISTVDSMIALDIDPLENTDFRVLELYSQKELRSSNVFDLEEIMREFNSYKQRVKYVEDKVVDPLPPYLKGLDDLMSGLGAAGKAVGVAIGAVGGAVASVVEGVATFLKNPFGAFTIILVAIAVVIITYLIYTRQRRLCTQPLQNLFPYLVSADGTTVTSGSTKDTSLQAPPSYEESVYNSGRKGPGPPSSDASTAAPPYTNEQAYQMLLALARLDAEQRAQQNGTDSLDGRTGTQDKGQKPNLLDRLRHRKNGYRHLKDSDEEENVGTGSSGVSKGEELFTGVVPILVELDGDVNGHKFSVRGEGEGDATNGKLTLKFICTTGKLPVPWPTLVTTLTYGVQCFSRYPDHMKQHDFFKSAMPEGYVQERTISFKDDGTYKTRAEVKFEGDTLVNRIELKGIDFKEDGNILGHKLEYNFNSHNVYITADKQKNGIKANFKIRHNVEDGSVQLADHYQQNTPIGDGPVLLPDNHYLSTQSKLSKDPNEKRDHMVLLEFVTAAGITLGMDELYK

SEQ ID NO: 11 - protein, 1080 aa, synthetic construct
  source 1..1080: note = EBV gB-sfEGFP used as transfected GFP-fusion; note = based on Uniprot P03188 (22-857) and GenBank MH644049.1 (2-238)
  REGION 1..836: note = EBV gB (22-857)
  REGION 844..1080: note = sfEGFP (2-238)
AQTPEQPAPPATTVQPTATRQQTSFPFRVCELSSHGDLFRFSSDIQCPSFGTRENHTEGLLMVFKDNIIPYSFKVRSYTKIVTNILIYNGWYADSVTNRHEEKFSVDSYETDQMDTIYQCYNAVKMTKDGLTRVYVDRDGVNITVNLKPTGGLANGVRRYASQTELYDAPGWLIWTYRTRTTVNCLITDMMAKSNSPFDFFVTTTGQTVEMSPFYDGKNKETFHERADSFHVRTNYKIVDYDNRGTNPQGERRAFLDKGTYTLSWKLENRTAYCPLQHWQTFDSTIATETGKSIHFVTDEGTSSFVTNTTVGIELPDAFKCIEEQVNKTMHEKYEAVQDRYTKGQEAITYFITSGGLLLAWLPLTPRSLATVKNLTELTTPTSSPPSSPSPPAPSAARGSTPAAVLRRRRRDAGNATTPVPPTAPGKSLGTLNNPATVQIQFAYDSLRRQINRMLGDLARAWCLEQKRQNMVLRELTKINPTTVMSSIYGKAVAAKRLGDVISVSQCVPVNQATVTLRKSMRVPGSETMCYSRPLVSFSFINDTKTYEGQLGTDNEIFLTKKMTEVCQATSQYYFQSGNEIHVYNDYHHFKTIELDGIATLQTFISLNTSLIENIDFASLELYSRDEQRASNVFDLEGIFREYNFQAQNIAGLRKDLDNAVSNGRNQFVDGLGELMDSLGSVGQSITNLVSTVGGLFSSLVSGFISFFKNPFGGMLILVLVAGVVILVISLTRRTRQMSQQPVQMLYPGIDELAQQHASGEGPGINPISKTELQAIMLALHEQNQEQKRAAQRAAGPSVASRALQAARDRFPGLRRRRYHDPETAAALLGEAETEFGTGSSGVSKGEELFTGVVPILVELDGDVNGHKFSVRGEGEGDATNGKLTLKFICTTGKLPVPWPTLVTTLTYGVQCFSRYPDHMKQHDFFKSAMPEGYVQERTISFKDDGTYKTRAEVKFEGDTLVNRIELKGIDFKEDGNILGHKLEYNFNSHNVYITADKQKNGIKANFKIRHNVEDGSVQLADHYQQNTPIGDGPVLLPDNHYLSTQSKLSKDPNEKRDHMVLLEFVTAAGITLGMDELYK

SEQ ID NO: 12 - protein, 738 aa, synthetic construct
  source 1..738: note = VSV G-sfEGFP used as transfected GFP-fusion; note = based on Uniprot B7UCZ5 (17-511) and GenBank MH644049.1 (2-238)
  REGION 1..495: note = VSV G (17-511)
  REGION 502..738: note = sfEGFP (2-238)
KFTIVFPHNQKGNWKNVPSNYHYCPSSSDLNWHNDLIGTALQVKMPKSHKAIQADGWMCHASKWVTTCDFRWYGPKYITHSIRSFTPSVEQCKESIEQTKQGTWLNPGFPPQSCGYATVTDAEAVIVQVTPHHVLVDEYTGEWVDSQFINGKCSNYICPTVHNSTTWHSDYKVKGLCDSNLISMDITFFSEDGELSSLGKEGTGFRSNYFAYETGGKACKMQYCKHWGVRLPSGVWFEMADKDLFAAARFPECPEGSSISAPSQTSVDVSLIQDVERILDYSLCQETWSKIRAGLPISPVDLSYLAPKNPGTGPAFTIINGTLKYFETRYIRVDIAAPILSRMVGMISGTTTERELWDDWAPYEDVEIGPNGVLRTSSGYKFPLYMIGHGMLDSDLHLSSKAQVFEHPHIQDAASQLPDDESLFFGDTGLSKNPIELVEGWFSSWKSSIASFFFIIGLIIGLFLVLRVGIHLCIKLKHTKKRQIYTDIEMNRLGKQLGSSVSKGEELFTGVVPILVELDGDVNGHKFSVRGEGEGDATNGKLTLKFICTTGKLPVPWPTLVTTLTYGVQCFSRYPDHMKQHDFFKSAMPEGYVQERTISFKDDGTYKTRAEVKFEGDTLVNRIELKGIDFKEDGNILGHKLEYNFNSHNVYITADKQKNGIKANFKIRHNVEDGSVQLADHYQQNTPIGDGPVLLPDNHYLSTQSKLSKDPNEKRDHMVLLEFVTAAGITLGMDELYK

SEQ ID NO: 13 - protein, 117 aa, synthetic construct
  source 1..117: note = Nb1_gbHSV (1-119) VHH sequence
  REGION 26..37: note = CDR1
  REGION 52..59: note = CDR2
  REGION 98..106: note = CDR3
  REGION 1: note = part of Nb1_gbHSV paratope
  REGION 26..29: note = part of Nb1_gbHSV paratope
  REGION 32: note = part of Nb1_gbHSV paratope
  REGION 34..35: note = part of Nb1_gbHSV paratope
  REGION 39: note = part of Nb1_gbHSV paratope
  REGION 49: note = part of Nb1_gbHSV paratope
  REGION 52: note = part of Nb1_gbHSV paratope
  REGION 54..56: note = part of Nb1_gbHSV paratope
  REGION 58..61: note = part of Nb1_gbHSV paratope
  REGION 66: note = part of Nb1_gbHSV paratope
  REGION 100..104: note = part of Nb1_gbHSV paratope
QVQLVESGGGSVQPGGSLRLSCAASASGRLSMSGALGWYRQVQGKSRELVATITDRSSTNYADSVKGRFTISIDDAENTMYLQMNSLKPEDTGVYYCNARWRGMNVWGKGTRVTVSS

SEQ ID NO: 14 - protein, 12 aa, synthetic construct
  source 1..12: note = Nb1_gbHSV_CDR1 (26-37)
ASGRLSMSGALG

SEQ ID NO: 15 - protein, 8 aa, synthetic construct
  source 1..8: note = Nb1_gbHSV_CDR2 (52-59)
TITDRSST

SEQ ID NO: 16 - protein, 9 aa, synthetic construct
  source 1..9: note = Nb1_gbHSV_CDR3 (98-106)
NARWRGMNV

SEQ ID NO: 17 - protein, 117 aa, synthetic construct
  source 1..117: note = Nb2_gbHSV (1-117) VHH sequence
  REGION 26..37: note = CDR1
  REGION 52..59: note = CDR2
  REGION 96..106: note = CDR3
QVQLVESGGGLVQPGGSLRLSCAASGVTFSSSVMSWHRQAPGQQREFVASITSAGVTDYADSVKGRATISRDNAQNTVYLQMNSLKPEDTAVYYCSAVPRPYQLQYWGQGTRVTVSS

SEQ ID NO: 18 - protein, 12 aa, synthetic construct
  source 1..12: note = Nb2_gbHSV_CDR1 (26-37)
ASGVTFSSSVMS

SEQ ID NO: 19 - protein, 9 aa, synthetic construct
  source 1..9: note = Nb2_gbHSV_CDR2 (52-59)
SITSAGVTD

SEQ ID NO: 20 - protein, 11 aa, synthetic construct
  source 1..11: note = Nb2_gbHSV_CDR3 (96-106)
SAVPRPYQLQY